European Patent Application EP 4 446 416 A2, published October 16, 2024. Title: CHIMERIC ENZYME AND METHOD FOR PRODUCING TERMINAL ALKENES. Applicant: CNPEM - CENTRO NACIONAL DE PESQUISA EM ENERGIA E MATERIAIS. The sequence listing filed with the application follows.

SEQUENCE LISTING (8 sequences)

SEQ ID NO: 1 - protein, 429 aa, Rothia nasimurium
MNIAPVKNLLNDQLPNFIKQGYLFMSHQRRKAGVPADSNCPVTFPVLGGRATLIRGEEAVDFFYDESKISRNGAMPTAIQGPLFGDGAVHTLDGQAHKVRKSAMAAMAYDDERVEAFRGFVEEEMKALIERWKTNPGNIYDDVAVAYGRAAFRWAGVPASDRELNKRATQMSHLLDTFGEVKQNVLSWMDRRKLDAWAEDLIKKVRSGELTVDPDSVVRHMADLRDEKGELVTAKLAGIELQNLTRPTVAVSRFAAFAAVAMVENPEWAAKVKNAVEDADGRLVNIPEAVAFAQETRRKYPFVPMLPAMVKEDTELSGCPIQKGQRVFLDVLGTNNSPQLWNNPGEFNPQRFLDTPDYESIKGFIPQGGGDVLTGHRCPGEKIAVAALSSTVAALSADNVTISQETEDTTFSMTQLLTRPRTGVRVTVS

SEQ ID NO: 2 - protein, 418 aa, Streptomyces sp.
MSDITVTNWAGNITYTAKELLRPHSLDALRALVADSARVRVLGSGHSFNEIAEPGDGGVLLSLAGLPSVVDVDTAARTVRVGGGVRYAELARVVHARGLALPNMASLPHISVAGSVATGTHGSGVGNGSLASVVREVELVTADGSTVVIARGDERFGGAVTSLGALGVVTSLTLDLEPAYEMEQHVFTELPLAGLDPATFETVMAAAYSVSLFTDWRAPGFRQVWLKRRTDRPLDGFPYAAPAAEKMHPVPGMPAVNCTEQFGVPGPWHERLPHFRAEFTPSSGAELQSEYLMPREHALAALHAMDAIRETLAPVLQTCEIRTVAADAQWLSPAYGRDTVAAHFTWVEDTAAVLPVVRRLEEALVPFAARPHWGKVFTVPAGELRALYPRLADFGALAGALDPAGKFTNAFVRGVLAG

SEQ ID NO: 3 - protein, 11 aa, unidentified
HSSGLVPRGSH

SEQ ID NO: 4 - protein, 13 aa, unidentified
DASAREATAKGSH

SEQ ID NO: 5 - protein, 858 aa, synthetic construct
MNIAPVKNLLNDQLPNFIKQGYLFMSHQRRKAGVPADSNCPVTFPVLGGRATLIRGEEAVDFFYDESKISRNGAMPTAIQGPLFGDGAVHTLDGQAHKVRKSAMAAMAYDDERVEAFRGFVEEEMKALIERWKTNPGNIYDDVAVAYGRAAFRWAGVPASDRELNKRATQMSHLLDTFGEVKQNVLSWMDRRKLDAWAEDLIKKVRSGELTVDPDSVVRHMADLRDEKGELVTAKLAGIELQNLTRPTVAVSRFAAFAAVAMVENPEWAAKVKNAVEDADGRLVNIPEAVAFAQETRRKYPFVPMLPAMVKEDTELSGCPIQKGQRVFLDVLGTNNSPQLWNNPGEFNPQRFLDTPDYESIKGFIPQGGGDVLTGHRCPGEKIAVAALSSTVAALSADNVTISQETEDTTFSMTQLLTRPRTGVRVTVSHSSGLVPRGSHMSDITVTNWAGNITYTAKELLRPHSLDALRALVADSARVRVLGSGHSFNEIAEPGDGGVLLSLAGLPSVVDVDTAARTVRVGGGVRYAELARVVHARGLALPNMASLPHISVAGSVATGTHGSGVGNGSLASVVREVELVTADGSTVVIARGDERFGGAVTSLGALGVVTSLTLDLEPAYEMEQHVFTELPLAGLDPATFETVMAAAYSVSLFTDWRAPGFRQVWLKRRTDRPLDGFPYAAPAAEKMHPVPGMPAVNCTEQFGVPGPWHERLPHFRAEFTPSSGAELQSEYLMPREHALAALHAMDAIRETLAPVLQTCEIRTVAADAQWLSPAYGRDTVAAHFTWVEDTAAVLPVVRRLEEALVPFAARPHWGKVFTVPAGELRALYPRLADFGALAGALDPAGKFTNAFVRGVLAG

SEQ ID NO: 6 - protein, 860 aa, synthetic construct
MNIAPVKNLLNDQLPNFIKQGYLFMSHQRRKAGVPADSNCPVTFPVLGGRATLIRGEEAVDFFYDESKISRNGAMPTAIQGPLFGDGAVHTLDGQAHKVRKSAMAAMAYDDERVEAFRGFVEEEMKALIERWKTNPGNIYDDVAVAYGRAAFRWAGVPASDRELNKRATQMSHLLDTFGEVKQNVLSWMDRRKLDAWAEDLIKKVRSGELTVDPDSVVRHMADLRDEKGELVTAKLAGIELQNLTRPTVAVSRFAAFAAVAMVENPEWAAKVKNAVEDADGRLVNIPEAVAFAQETRRKYPFVPMLPAMVKEDTELSGCPIQKGQRVFLDVLGTNNSPQLWNNPGEFNPQRFLDTPDYESIKGFIPQGGGDVLTGHRCPGEKIAVAALSSTVAALSADNVTISQETEDTTFSMTQLLTRPRTGVRVTGSDASAREATAKGSHMSDITVTNWAGNITYTAKELLRPHSLDALRALVADSARVRVLGSGHSFNEIAEPGDGGVLLSLAGLPSVVDVDTAARTVRVGGGVRYAELARVVHARGLALPNMASLPHISVAGSVATGTHGSGVGNGSLASVVREVELVTADGSTVVIARGDERFGGAVTSLGALGVVTSLTLDLEPAYEMEQHVFTELPLAGLDPATFETVMAAAYSVSLFTDWRAPGFRQVWLKRRTDRPLDGFPYAAPAAEKMHPVPGMPAVNCTEQFGVPGPWHERLPHFRAEFTPSSGAELQSEYLMPREHALAALHAMDAIRETLAPVLQTCEIRTVAADAQWLSPAYGRDTVAAHFTWVEDTAAVLPVVRRLEEALVPFAARPHWGKVFTVPAGELRALYPRLADFGALAGALDPAGKFTNAFVRGVLAG

SEQ ID NO: 7 - DNA, 2574 bp, synthetic construct
  source 1..2574: mol_type = other DNA
atgaacatcgcacccgtaaaaaatcttttgaatgaccagctgcccaatttcattaagcagggctacctttttatgtcccaccagcgccgtaaggccggggttcccgcagattccaactgccccgttaccttccccgtcctgggaggaagggccaccctaattcgaggtgaagaggccgtagatttcttctacgatgagtctaaaattagccgtaacggtgctatgcccaccgccattcaggggccgctctttggcgacggtgccgtgcacaccctcgacggtcaggcgcataaggttcgtaagtctgccatggctgccatggcctatgacgacgagcgggtagaggctttcaggggcttcgtcgaagaagaaatgaaggccctcattgagcggtggaagaccaaccccggcaacatctacgatgacgttgctgtggcctacggtcgcgctgccttccgctgggccggggtgccagcctccgaccgcgaactcaacaagcgagccacccagatgagccacctgctcgacacgttcggcgaggtcaagcagaacgtgctctcctggatggaccgccgcaaactcgatgcctgggccgaagacctcatcaaaaaggtacgctcgggcgaactcacggttgaccctgactctgtggtgcgccacatggcagatttgcgtgatgagaagggcgaactggtcaccgccaagctggccggtatcgaattgcagaacctgactcgccctaccgtggcggtctcccgctttgcagccttcgcagctgtagccatggtcgaaaaccccgagtgggccgccaaggtcaagaatgctgttgaggacgccgacggccgcctagtcaatatccccgaagctgttgccttcgcccaggagacccgccgcaagtaccccttcgtccccatgcttcccgctatggttaaggaagatactgaactttcgggttgcccgattcagaagggccagcgggtgttccttgatgttttaggtacaaacaactcaccccaactctggaacaaccccggtgaattcaacccccagcgtttcttggataccccggactatgagtccattaagggtttcatccctcagggcggcggagacgtgctcaccggccaccgttgccccggcgagaagattgctgtggcggctctgtcttcaaccgttgcagcgctttcagctgataacgtcaccatctctcaagaaaccgaagacaccactttcagtatgacccagctactcacccgccccaggacgggcgtacgcgtaacagtcagccacagcagcggcctggtgccgcgcggcagccatatgtctgacatcaccgttaccaactgggctggtaacatcacctacaccgctaaagaactgctgcgtccgcactctctggacgctctgcgtgctctggttgctgactctgctcgtgttcgtgttctgggttctggtcactctttcaacgaaatcgctgaaccgggtgacggtggtgttctgctgtctctggctggtctgccgtctgttgttgacgttgacaccgctgctcgtaccgttcgtgttggtggtggtgttcgttacgctgaactggctcgtgttgttcacgctcgtggtctggctctgccgaacatggcttctctgccgcacatctctgttgctggttctgttgctaccggtacccacggttctggtgttggtaacggttctctggcttctgttgttcgtgaagttgaactggttaccgctgacggttctaccgttgttatcgctcgtggtgacgaacgtttcggtggtgctgttacctctctgggtgctctgggtgttgttacctctctgaccctggacctggaaccggcttacgaaatggaacagcacgttttcaccgaactgccgctggctggtctggacccggctaccttcgaaaccgttatggctgctgcttactctgtttctctgttcaccgactggcgtgctccgggtttccgtcaggtttggctgaaacgtcgtaccgaccgtccgctggacggtttcccgtacgctgctccggctgctgaaaaaatgcacccggttccgggtatgccggctgttaactgcaccgaacagttcggtgttccgggtccgtggcacgaacgtctgccgcacttccgtgctgaattcaccccgtcttctggtgctgaactgcagtctgaatacctgatgccgcgtgaacacgctctggctgctctgcacgctatggacgctatccgtgaaaccctggctccggttctgcagacctgcgaaatccgtaccgttgctgctgacgctcagtggctgtctccggcttacggtcgtgacaccgttgctgctcacttcacctgggttgaagacaccgctgctgttctgccggttgttcgtcgtctggaagaagctctggttccgttcgctgctcgtccgcactggggtaaagttttcaccgttccggctggtgaactgcgtgctctgtacccgcgtctggctgacttcggtgctctggctggtgctctggacccggctggtaaattcaccaacgctttcgttcgtggtgttctggctggt

SEQ ID NO: 8 - DNA, 2580 bp, synthetic construct
  source 1..2580: mol_type = other DNA
atgaacatcgcacccgtaaaaaatcttttgaatgaccagctgcccaatttcattaagcagggctacctttttatgtcccaccagcgccgtaaggccggggttcccgcagattccaactgccccgttaccttccccgtcctgggaggaagggccaccctaattcgaggtgaagaggccgtagatttcttctacgatgagtctaaaattagccgtaacggtgctatgcccaccgccattcaggggccgctctttggcgacggtgccgtgcacaccctcgacggtcaggcgcataaggttcgtaagtctgccatggctgccatggcctatgacgacgagcgggtagaggctttcaggggcttcgtcgaagaagaaatgaaggccctcattgagcggtggaagaccaaccccggcaacatctacgatgacgttgctgtggcctacggtcgcgctgccttccgctgggccggggtgccagcctccgaccgcgaactcaacaagcgagccacccagatgagccacctgctcgacacgttcggcgaggtcaagcagaacgtgctctcctggatggaccgccgcaaactcgatgcctgggccgaagacctcatcaaaaaggtacgctcgggcgaactcacggttgaccctgactctgtggtgcgccacatggcagatttgcgtgatgagaagggcgaactggtcaccgccaagctggccggtatcgaattgcagaacctgactcgccctaccgtggcggtctcccgctttgcagccttcgcagctgtagccatggtcgaaaaccccgagtgggccgccaaggtcaagaatgctgttgaggacgccgacggccgcctagtcaatatccccgaagctgttgccttcgcccaggagacccgccgcaagtaccccttcgtccccatgcttcccgctatggttaaggaagatactgaactttcgggttgcccgattcagaagggccagcgggtgttccttgatgttttaggtacaaacaactcaccccaactctggaacaaccccggtgaattcaacccccagcgtttcttggataccccggactatgagtccattaagggtttcatccctcagggcggcggagacgtgctcaccggccaccgttgccccggcgagaagattgctgtggcggctctgtcttcaaccgttgcagcgctttcagctgataacgtcaccatctctcaagaaaccgaagacaccactttcagtatgacccagctactcacccgccccaggacgggcgtacgcgtaacaggcagcgacgcttctgctcgtgaagctaccgctaaaggcagccatatgtctgacatcaccgttaccaactgggctggtaacatcacctacaccgctaaagaactgctgcgtccgcactctctggacgctctgcgtgctctggttgctgactctgctcgtgttcgtgttctgggttctggtcactctttcaacgaaatcgctgaaccgggtgacggtggtgttctgctgtctctggctggtctgccgtctgttgttgacgttgacaccgctgctcgtaccgttcgtgttggtggtggtgttcgttacgctgaactggctcgtgttgttcacgctcgtggtctggctctgccgaacatggcttctctgccgcacatctctgttgctggttctgttgctaccggtacccacggttctggtgttggtaacggttctctggcttctgttgttcgtgaagttgaactggttaccgctgacggttctaccgttgttatcgctcgtggtgacgaacgtttcggtggtgctgttacctctctgggtgctctgggtgttgttacctctctgaccctggacctggaaccggcttacgaaatggaacagcacgttttcaccgaactgccgctggctggtctggacccggctaccttcgaaaccgttatggctgctgcttactctgtttctctgttcaccgactggcgtgctccgggtttccgtcaggtttggctgaaacgtcgtaccgaccgtccgctggacggtttcccgtacgctgctccggctgctgaaaaaatgcacccggttccgggtatgccggctgttaactgcaccgaacagttcggtgttccgggtccgtggcacgaacgtctgccgcacttccgtgctgaattcaccccgtcttctggtgctgaactgcagtctgaatacctgatgccgcgtgaacacgctctggctgctctgcacgctatggacgctatccgtgaaaccctggctccggttctgcagacctgcgaaatccgtaccgttgctgctgacgctcagtggctgtctccggcttacggtcgtgacaccgttgctgctcacttcacctgggttgaagacaccgctgctgttctgccggttgttcgtcgtctggaagaagctctggttccgttcgctgctcgtccgcactggggtaaagttttcaccgttccggctggtgaactgcgtgctctgtacccgcgtctggctgacttcggtgctctggctggtgctctggacccggctggtaaattcaccaacgctttcgttcgtggtgttctggctggt